European Patent Application EP 4 339 291 A1, published March 20, 2024. Title: LENTIVIRAL VECTORS AND USES THEREOF. Applicant: Centro de Investigaciones Energéticas, Medioambientales y Tecnológicas, O.A., M.P. (CIEMAT) Consorcio Centro de Investigación Biomédica en Red, M.P. (CIBER) Fundación Instituto de Investigación Sanitaria Fundación Jiménez Díaz (FIIS-FJD). Université Libre de Bruxelles Fundación para la Investigación Biomédica del Hospital Infantil Universitario Niño Jesús. The sequence listing filed with the application follows.

SEQUENCE LISTING (39 sequences)

SEQ ID NO: 1 - DNA, 780 bp, Artificial Sequence
  5’ LTR
gacattgattattgactagttattaatagtaatcaattacggggtcattagttcatagcccatatatggagttccgcgttacataacttacggtaaatggcccgcctggctgaccgcccaacgacccccgcccattgacgtcaataatgacgtatgttcccatagtaacgccaatagggactttccattgacgtcaatgggtggagtatttacggtaaactgcccacttggcagtacatcaagtgtatcatatgccaagtacgccccctattgacgtcaatgacggtaaatggcccgcctggcattatgcccagtacatgaccttatgggactttcctacttggcagtacatctacgtattagtcatcgctattaccatggtgatgcggttttggcagtacatcaatgggcgtggatagcggtttgactcacggggatttccaagtctccaccccattgacgtcaatgggagtttgttttggcaccaaaatcaacgggactttccaaaatgtcgtaacaactccgccccattgacgcaaatgggcggtaggcgtgtacggtgggaggtctatataagcagagctcgtttagtgaaccggggtctctctggttagaccagatctgagcctgggagctctctggctaactagggaacccactgcttaagcctcaataaagcttgccttgagtgcttcaagtagtgtgtgcccgtctgttgtgtgactctggtaactagagatccctcagacccttttagtcagtgtggaaaatctctagcag

SEQ ID NO: 2 - DNA, 584 bp, Artificial Sequence
  Chimeric CMV promoter
gacattgattattgactagttattaatagtaatcaattacggggtcattagttcatagcccatatatggagttccgcgttacataacttacggtaaatggcccgcctggctgaccgcccaacgacccccgcccattgacgtcaataatgacgtatgttcccatagtaacgccaatagggactttccattgacgtcaatgggtggagtatttacggtaaactgcccacttggcagtacatcaagtgtatcatatgccaagtacgccccctattgacgtcaatgacggtaaatggcccgcctggcattatgcccagtacatgaccttatgggactttcctacttggcagtacatctacgtattagtcatcgctattaccatggtgatgcggttttggcagtacatcaatgggcgtggatagcggtttgactcacggggatttccaagtctccaccccattgacgtcaatgggagtttgttttggcaccaaaatcaacgggactttccaaaatgtcgtaacaactccgccccattgacgcaaatgggcggtaggcgtgtacggtgggaggtctatataagcagagct

SEQ ID NO: 3 - DNA, 380 bp, Artificial Sequence
  CMV enhancer
gacattgattattgactagttattaatagtaatcaattacggggtcattagttcatagcccatatatggagttccgcgttacataacttacggtaaatggcccgcctggctgaccgcccaacgacccccgcccattgacgtcaataatgacgtatgttcccatagtaacgccaatagggactttccattgacgtcaatgggtggagtatttacggtaaactgcccacttggcagtacatcaagtgtatcatatgccaagtacgccccctattgacgtcaatgacggtaaatggcccgcctggcattatgcccagtacatgaccttatgggactttcctacttggcagtacatctacgtattagtcatcgctattaccatg

SEQ ID NO: 4 - DNA, 204 bp, Artificial Sequence
  CMV promoter
gtgatgcggttttggcagtacatcaatgggcgtggatagcggtttgactcacggggatttccaagtctccaccccattgacgtcaatgggagtttgttttggcaccaaaatcaacgggactttccaaaatgtcgtaacaactccgccccattgacgcaaatgggcggtaggcgtgtacggtgggaggtctatataagcagagct

SEQ ID NO: 5 - DNA, 182 bp, Artificial Sequence
  RU5. Truncated 5' LTR without RU3
gggtctctctggttagaccagatctgagcctgggagctctctggctaactagggaacccactgcttaagcctcaataaagcttgccttgagtgcttcaagtagtgtgtgcccgtctgttgtgtgactctggtaactagagatccctcagacccttttagtcagtgtggaaaatctctagcag

SEQ ID NO: 6 - DNA, 18 bp, Artificial Sequence
  PBS SL123 (Primer Binding Site)
tggcgcccgaacagggac

SEQ ID NO: 7 - DNA, 126 bp, Artificial Sequence
  packaging signal
ctctctcgacgcaggactcggcttgctgaagcgcgcacggcaagaggcgaggggcggcgactggtgagtacgccaaaaattttgactagcggaggctagaaggagagagatgggtgcgagagcgtc

SEQ ID NO: 8 - DNA, 234 bp, Artificial Sequence
  RRE
aggagctttgttccttgggttcttgggagcagcaggaagcactatgggcgcagcgtcaatgacgctgacggtacaggccagacaattattgtctggtatagtgcagcagcagaacaatttgctgagggctattgaggcgcaacagcatctgttgcaactcacagtctggggcatcaagcagctccaggcaagaatcctggctgtggaaagatacctaaaggatcaacagctcct

SEQ ID NO: 9 - DNA, 118 bp, Artificial Sequence
  cPPT
ttttaaaagaaaaggggggattggggggtacagtgcaggggaaagaatagtagacataatagcaacagacatacaaactaaagaattacaaaaacaaattacaaaaattcaaaatttt

SEQ ID NO: 10 - DNA, 511 bp, Artificial Sequence
  Phosphoglicerate kinase promoter PGK
ggggttggggttgcgccttttccaaggcagccctgggtttgcgcagggacgcggctgctctgggcgtggttccgggaaacgcagcggcgccgaccctgggtctcgcacattcttcacgtccgttcgcagcgtcacccggatcttcgccgctacccttgtgggccccccggcgacgcttcctgctccgcccctaagtcgggaaggttccttgcggttcgcggcgtgccggacgtgacaaacggaagccgcacgtctcactagtaccctcgcagacggacagcgccagggagcaatggcagcgcgccgaccgcgatgggctgtggccaatagcggctgctcagcagggcgcgccgagagcagcggccgggaaggggcggtgcgggaggcggggtgtggggcggtagtgtgggccctgttcctgcccgcgcggtgttccgcattctgcaagcctccggagcgcacgtcggcagtcggctccctcgttgaccgaatcaccgacctctctccccag

SEQ ID NO: 11 - DNA, 251 bp, Artificial Sequence
  Elongation fator alpha short promoter (E1Fα(s))
atcatggctccggtgcccgtcagtgggcagagcgcacatcgcccacagtccccgagaagttggggggaggggtcggcaattgaaccggtgcctagagaaggtggcgcggggtaaactgggaaagtgatgtcgtgtactggctccgcctttttcccgagggtgggggagaaccgtatataagtgcagtagtcgccgtgaacgttctttttcgcaacgggtttgccgccagaacacaggtgtcgtgacgctcg

SEQ ID NO: 12 - DNA, 441 bp, Artificial Sequence
  Codon optimized version of RPS19  (CoRPS19)
atgcccggcgtgaccgtgaaggacgtgaaccagcaggagttcgtgagggccctggcagcctttctgaagaagagcggcaagctgaaggtgcccgagtgggtggacacagtgaagctggccaagcacaaggagctggccccttacgatgagaactggttctataccagggcagcctccacagcaaggcacctgtacctgaggggaggagcaggagtgggctctatgaccaagatctatggcggcaggcagcgcaatggcgtgatgccatctcactttagccggggcagcaagtccgtggcaaggagagtgctgcaggccctggagggcctgaagatggtggagaaggaccaggatggcggcagaaagctgacaccacagggacagcgggacctggatagaatcgcaggacaggtggcagcagccaataagaagcactgatag

SEQ ID NO: 13 - DNA, 589 bp, Artificial Sequence
  Mutated Wpre (Wpre*)
cgagcatcttaccgccatttattcccatatttgttctgtttttcttgatttgggtatacatttaaatgttaataaaacaaaatggtggggcaatcatttacatttttagggatatgtaattactagttcaggtgtattgccacaagacaaacatgttaagaaactttcccgttatttacgctctgttcctgttaatcaacctctggattacaaaatttgtgaaagattgactgatattcttaactatgttgctccttttacgctgtgtggatatgctgctttaatgcctctgtatcatgctattgcttcccgtacggctttcgttttctcctccttgtataaatcctggttgctgtctctttatgaggagttgtggcccgttgtccgtcaacgtggcgtggtgtgctctgtgtttgctgacgcaacccccactggctggggcattgccaccacctgtcaactcctttctgggactttcgctttccccctcccgatcgccacggcagaactcatcgccgcctgccttgcccgctgctggacaggggctaggttgctgggcactgataattccgtggtgttgtcggggaag

SEQ ID NO: 14 - DNA, 234 bp, Artificial Sequence
  3’ LTR: DR3RU5
tggaagggctaattcactcccaacgaagacaagatctgctttttgcttgtactgggtctctctggttagaccagatctgagcctgggagctctctggctaactagggaacccactgcttaagcctcaataaagcttgccttgagtgcttcaagtagtgtgtgcccgtctgttgtgtgactctggtaactagagatccctcagacccttttagtcagtgtggaaaatctctagca

SEQ ID NO: 15 - DNA, 54 bp, Artificial Sequence
  ΔU3
tggaagggctaattcactcccaacgaagacaagatctgctttttgcttgtactg

SEQ ID NO: 16 - DNA, 181 bp, Artificial Sequence
  RU5
ggtctctctggttagaccagatctgagcctgggagctctctggctaactagggaacccactgcttaagcctcaataaagcttgccttgagtgcttcaagtagtgtgtgcccgtctgttgtgtgactctggtaactagagatccctcagacccttttagtcagtgtggaaaatctctagcag

SEQ ID NO: 17 - DNA, 7821 bp, Artificial Sequence
  PGK.CoRPS19. Wpre*- LV sequence
gtgtttaaacctagatattgatagtctgatcggtcaacgtataatcgagtcctagcttttgcaaacatctatcaagagacaggatcagcaggaggctttcgcatgattgaacaagatggattgcacgcaggttctccggcggcttgggtggagaggctattcggctatgactgggcacaacagacaatcggctgctctgatgccgccgtgttccggctgtcagcgcaggggcgtccggttctttttgtcaagaccgacctgtccggtgccctgaatgaactgcaagacgaggcagcgcggctatcgtggctggcgacgacgggcgttccttgcgcggctgtgctcgacgttgtcactgaagcgggaagggactggctgctattgggcgaagtgccggggcaggatctcctgtcatctcaccttgctcctgccgagaaagtatccatcatggctgatgcaatgcggcggctgcatacgcttgatccggctacctgcccattcgaccaccaagcgaaacatcgcatcgagcgagcacgtactcggatggaagccggtcttgtcgatcaggatgatctggacgaagagcatcaggggctcgcgccagccgaactgttcgccaggctcaaggcgtctatgcccgacggcgaggatctcgtcgtgacccacggcgatgcctgcttgccgaatatcatggtggaaaatggccgcttttctggattcatcgactgtggccgtctgggtgtggcggaccgctatcaggacatagcgttggctacccgtgatattgctgaagagcttggcggcgaatgggctgaccgcttccttgtgctttacggtatcgccgcgcccgattcgcagcgcatcgccttctatcgccttcttgacgagttcttctgaccgattctaggtgcattggcgcagaaaaaaatgcctgatgcgacgctgcgcgtcttatactcccacatatgccagattcagcaacggatacggcttccccaacttgcccacttccatacgtgtcctccttaccagaaatttatccttaacgatcggacggggagtcaggcaactatggatgaacgaaatagacagatcgctgagataggtgcctcactgattaagcattggtaactgtcagaccaagtttactcatatatactttagattgatttaaaacttcatttttaatttaaaaggatctaggtgaagatcctttttgataatctcatgaccaaaatcccttaacgtgagttttcgttccactgagcgtcagaccccgtagaaaagatcaaaggatcttcttgagatcctttttttctgcgcgtaatctgctgcttgcaaacaaaaaaaccaccgctaccagcggtggtttgtttgccggatcaagagctaccaactctttttccgaaggtaactggcttcagcagagcgcagataccaaatactgtccttctagtgtagccgtagttaggccaccacttcaagaactctgtagcaccgcctacatacctcgctctgctaatcctgttaccagtggctgctgccagtggcgataagtcgtgtcttaccgggttggactcaagacgatagttaccggataaggcgcagcggtcgggctgaacggggggttcgtgcacacagcccagcttggagcgaacgacctacaccgaactgagatacctacagcgtgagctatgagaaagcgccacgcttcccgaagggagaaaggcggacaggtatccggtaagcggcagggtcggaacaggagagcgcacgagggagcttccagggggaaacgcctggtatctttatagtcctgtcgggtttcgccacctctgacttgagcgtcgatttttgtgatgctcgtcaggggggcggagcctatggaaaaacgccagcaacgcggcctttttacggttcctggccttttgctggccttttgctcacatgttctttcctgcgttatcccctgattctgtggataaccgtattaccgcctttgagtgagctgataccgctcgccgcagccgaacgaccgagcgcagcgagtcagtgagcgaggaagcggaagagcgcccaatacgcaaaccgcctctccccgcgcgttggccgattcattaatgcagctggcacgacaggtttcccgactggaaagcgggcagtgagcgcaacgcaattaatgtgagttagctcactcattaggcaccccaggctttacactttatgcttccggctcgtatgttgtgtggaattgtgagcggataacaatttcacacaggaaacagctatgaccatgattacgccaagcgcgcaattaaccctcactaaagggaacaaaagctggagctgcaagcttggccattgcatacgttgtatccatatcataatatgtacatttatattggctcatgtccaacattaccgccatgttgacattgattattgactagttattaatagtaatcaattacggggtcattagttcatagcccatatatggagttccgcgttacataacttacggtaaatggcccgcctggctgaccgcccaacgacccccgcccattgacgtcaataatgacgtatgttcccatagtaacgccaatagggactttccattgacgtcaatgggtggagtatttacggtaaactgcccacttggcagtacatcaagtgtatcatatgccaagtacgccccctattgacgtcaatgacggtaaatggcccgcctggcattatgcccagtacatgaccttatgggactttcctacttggcagtacatctacgtattagtcatcgctattaccatggtgatgcggttttggcagtacatcaatgggcgtggatagcggtttgactcacggggatttccaagtctccaccccattgacgtcaatgggagtttgttttggcaccaaaatcaacgggactttccaaaatgtcgtaacaactccgccccattgacgcaaatgggcggtaggcgtgtacggtgggaggtctatataagcagagctcgtttagtgaaccggggtctctctggttagaccagatctgagcctgggagctctctggctaactagggaacccactgcttaagcctcaataaagcttgccttgagtgcttcaagtagtgtgtgcccgtctgttgtgtgactctggtaactagagatccctcagacccttttagtcagtgtggaaaatctctagcagtggcgcccgaacagggacttgaaagcgaaagggaaaccagaggagctctctcgacgcaggactcggcttgctgaagcgcgcacggcaagaggcgaggggcggcgactggtgagtacgccaaaaattttgactagcggaggctagaaggagagagatgggtgcgagagcgtcagtattaagcgggggagaattagatcgcgatgggaaaaaattcggttaaggccagggggaaagaaaaaatataaattaaaacatatagtatgggcaagcagggagctagaacgattcgcagttaatcctggcctgttagaaacatcagaaggctgtagacaaatactgggacagctacaaccatcccttcagacaggatcagaagaacttagatcattatataatacagtagcaaccctctattgtgtgcatcaaaggatagagataaaagacaccaaggaagctttagacaagatagaggaagagcaaaacaaaagtaagaccaccgcacagcaagcggccgctgatcttcagacctggaggaggagatatgagggacaattggagaagtgaattatataaatataaagtagtaaaaattgaaccattaggagtagcacccaccaaggcaaagagaagagtggtgcagagagaaaaaagagcagtgggaataggagctttgttccttgggttcttgggagcagcaggaagcactatgggcgcagcgtcaatgacgctgacggtacaggccagacaattattgtctggtatagtgcagcagcagaacaatttgctgagggctattgaggcgcaacagcatctgttgcaactcacagtctggggcatcaagcagctccaggcaagaatcctggctgtggaaagatacctaaaggatcaacagctcctggggatttggggttgctctggaaaactcatttgcaccactgctgtgccttggaatgctagttggagtaataaatctctggaacagatttggaatcacacgacctggatggagtgggacagagaaattaacaattacacaagcttaatacactccttaattgaagaatcgcaaaaccagcaagaaaagaatgaacaagaattattggaattagataaatgggcaagtttgtggaattggtttaacataacaaattggctgtggtatataaaattattcataatgatagtaggaggcttggtaggtttaagaatagtttttgctgtactttctatagtgaatagagttaggcagggatattcaccattatcgtttcagacccacctcccaaccccgaggggacccgacaggcccgaaggaatagaagaagaaggtggagagagagacagagacagatccattcgattagtgaacggatctcgacggtatcggttaacttttaaaagaaaaggggggattggggggtacagtgcaggggaaagaatagtagacataatagcaacagacatacaaactaaagaattacaaaaacaaattacaaaaattcaaaattttatcgatcacgagactagcctcgagaagcttgatatcgaattccacggggttggggttgcgccttttccaaggcagccctgggtttgcgcagggacgcggctgctctgggcgtggttccgggaaacgcagcggcgccgaccctgggtctcgcacattcttcacgtccgttcgcagcgtcacccggatcttcgccgctacccttgtgggccccccggcgacgcttcctgctccgcccctaagtcgggaaggttccttgcggttcgcggcgtgccggacgtgacaaacggaagccgcacgtctcactagtaccctcgcagacggacagcgccagggagcaatggcagcgcgccgaccgcgatgggctgtggccaatagcggctgctcagcagggcgcgccgagagcagcggccgggaaggggcggtgcgggaggcggggtgtggggcggtagtgtgggccctgttcctgcccgcgcggtgttccgcattctgcaagcctccggagcgcacgtcggcagtcggctccctcgttgaccgaatcaccgacctctctccccagggggatccgtcgacacaccggtatgcccggcgtgaccgtgaaggacgtgaaccagcaggagttcgtgagggccctggcagcctttctgaagaagagcggcaagctgaaggtgcccgagtgggtggacacagtgaagctggccaagcacaaggagctggccccttacgatgagaactggttctataccagggcagcctccacagcaaggcacctgtacctgaggggaggagcaggagtgggctctatgaccaagatctatggcggcaggcagcgcaatggcgtgatgccatctcactttagccggggcagcaagtccgtggcaaggagagtgctgcaggccctggagggcctgaagatggtggagaaggaccaggatggcggcagaaagctgacaccacagggacagcgggacctggatagaatcgcaggacaggtggcagcagccaataagaagcactgataggatcccatctagaggatcccccgggctgcaggaattcgagcatcttaccgccatttattcccatatttgttctgtttttcttgatttgggtatacatttaaatgttaataaaacaaaatggtggggcaatcatttacatttttagggatatgtaattactagttcaggtgtattgccacaagacaaacatgttaagaaactttcccgttatttacgctctgttcctgttaatcaacctctggattacaaaatttgtgaaagattgactgatattcttaactatgttgctccttttacgctgtgtggatatgctgctttaatgcctctgtatcatgctattgcttcccgtacggctttcgttttctcctccttgtataaatcctggttgctgtctctttatgaggagttgtggcccgttgtccgtcaacgtggcgtggtgtgctctgtgtttgctgacgcaacccccactggctggggcattgccaccacctgtcaactcctttctgggactttcgctttccccctcccgatcgccacggcagaactcatcgccgcctgccttgcccgctgctggacaggggctaggttgctgggcactgataattccgtggtgttgtcggggaagggcctgctgccggctctgcggcctcttccgcgtcttcgccttcgccctcagacgagtcggatctccctttgggccgcctccccgcctggaattcgagctcggtacctttaagaccaatgacttacaaggcagctgtagatcttagccactttttaaaagaaaaggggggactggaagggctaattcactcccaacgaagacaagatctgctttttgcttgtactgggtctctctggttagaccagatctgagcctgggagctctctggctaactagggaacccactgcttaagcctcaataaagcttgccttgagtgcttcaagtagtgtgtgcccgtctgttgtgtgactctggtaactagagatccctcagacccttttagtcagtgtggaaaatctctagcagtagtagttcatgtcatcttattattcagtatttataacttgcaaagaaatgaatatcagagagtgagaggaacttgtttattgcagcttataatggttacaaataaagcaatagcatcacaaatttcacaaataaagcatttttttcactgcattctagttgtggtttgtccaaactcatcaatgtatcttatcatgtctggctctagctatcccgcccctaactccgcccatcccgcccctaactccgcccatcccgcccctaactccgcccagttccgcccattctccgccccatggctgactaattttttttatttatgcagaggccgaggccgcctcggcctctgagctattccagaagtagtgaggaggcttttttggaggcctagggacgtacccaattcgccctatagtgagtcgtattacgcgcgctcactggccgtcgttttacaacgtcgtgactgggaaaaccctggcgttacccaacttaatcgccttgcagcacatccccctttcgccagctggcgtaatagcgaagaggcccgcaccgatcgcccttcccaacagttgcgcagcctgaatggcgaatgggacgcgccctgtagcggcgcattaagcgcggcgggtgtggtggttacgcgcagcgtgaccgctacacttgccagcgccctagcgcccgctcctttcgctttcttcccttcctttctcgccacgttcgccggctttccccgtcaagctctaaatcgggggctccctttagggttccgatttagtgctttacggcacctcgaccccaaaaaacttgattagggtgatggttcacgtagtgggccatcgccctgatagacggtttttcgccctttgacgttggagtccacgttctttaatagtggactcttgttccaaactggaacaacactcaaccctatctcggtctattcttttgatttataagggattttgccgatttcggcctattggttaaaaaatgagctgatttaacaaaaatttaacgcgaattttaacaaaatcgttccctcaggacgtc

SEQ ID NO: 18 - DNA, 7540 bp, Artificial Sequence
  EF1α(s).CoRPS19. Wpre*- LV sequence
gtgtttaaacctagatattgatagtctgatcggtcaacgtataatcgagtcctagcttttgcaaacatctatcaagagacaggatcagcaggaggctttcgcatgattgaacaagatggattgcacgcaggttctccggcggcttgggtggagaggctattcggctatgactgggcacaacagacaatcggctgctctgatgccgccgtgttccggctgtcagcgcaggggcgtccggttctttttgtcaagaccgacctgtccggtgccctgaatgaactgcaagacgaggcagcgcggctatcgtggctggcgacgacgggcgttccttgcgcggctgtgctcgacgttgtcactgaagcgggaagggactggctgctattgggcgaagtgccggggcaggatctcctgtcatctcaccttgctcctgccgagaaagtatccatcatggctgatgcaatgcggcggctgcatacgcttgatccggctacctgcccattcgaccaccaagcgaaacatcgcatcgagcgagcacgtactcggatggaagccggtcttgtcgatcaggatgatctggacgaagagcatcaggggctcgcgccagccgaactgttcgccaggctcaaggcgtctatgcccgacggcgaggatctcgtcgtgacccacggcgatgcctgcttgccgaatatcatggtggaaaatggccgcttttctggattcatcgactgtggccgtctgggtgtggcggaccgctatcaggacatagcgttggctacccgtgatattgctgaagagcttggcggcgaatgggctgaccgcttccttgtgctttacggtatcgccgcgcccgattcgcagcgcatcgccttctatcgccttcttgacgagttcttctgaccgattctaggtgcattggcgcagaaaaaaatgcctgatgcgacgctgcgcgtcttatactcccacatatgccagattcagcaacggatacggcttccccaacttgcccacttccatacgtgtcctccttaccagaaatttatccttaacgatcggacggggagtcaggcaactatggatgaacgaaatagacagatcgctgagataggtgcctcactgattaagcattggtaactgtcagaccaagtttactcatatatactttagattgatttaaaacttcatttttaatttaaaaggatctaggtgaagatcctttttgataatctcatgaccaaaatcccttaacgtgagttttcgttccactgagcgtcagaccccgtagaaaagatcaaaggatcttcttgagatcctttttttctgcgcgtaatctgctgcttgcaaacaaaaaaaccaccgctaccagcggtggtttgtttgccggatcaagagctaccaactctttttccgaaggtaactggcttcagcagagcgcagataccaaatactgtccttctagtgtagccgtagttaggccaccacttcaagaactctgtagcaccgcctacatacctcgctctgctaatcctgttaccagtggctgctgccagtggcgataagtcgtgtcttaccgggttggactcaagacgatagttaccggataaggcgcagcggtcgggctgaacggggggttcgtgcacacagcccagcttggagcgaacgacctacaccgaactgagatacctacagcgtgagctatgagaaagcgccacgcttcccgaagggagaaaggcggacaggtatccggtaagcggcagggtcggaacaggagagcgcacgagggagcttccagggggaaacgcctggtatctttatagtcctgtcgggtttcgccacctctgacttgagcgtcgatttttgtgatgctcgtcaggggggcggagcctatggaaaaacgccagcaacgcggcctttttacggttcctggccttttgctggccttttgctcacatgttctttcctgcgttatcccctgattctgtggataaccgtattaccgcctttgagtgagctgataccgctcgccgcagccgaacgaccgagcgcagcgagtcagtgagcgaggaagcggaagagcgcccaatacgcaaaccgcctctccccgcgcgttggccgattcattaatgcagctggcacgacaggtttcccgactggaaagcgggcagtgagcgcaacgcaattaatgtgagttagctcactcattaggcaccccaggctttacactttatgcttccggctcgtatgttgtgtggaattgtgagcggataacaatttcacacaggaaacagctatgaccatgattacgccaagcgcgcaattaaccctcactaaagggaacaaaagctggagctgcaagcttggccattgcatacgttgtatccatatcataatatgtacatttatattggctcatgtccaacattaccgccatgttgacattgattattgactagttattaatagtaatcaattacggggtcattagttcatagcccatatatggagttccgcgttacataacttacggtaaatggcccgcctggctgaccgcccaacgacccccgcccattgacgtcaataatgacgtatgttcccatagtaacgccaatagggactttccattgacgtcaatgggtggagtatttacggtaaactgcccacttggcagtacatcaagtgtatcatatgccaagtacgccccctattgacgtcaatgacggtaaatggcccgcctggcattatgcccagtacatgaccttatgggactttcctacttggcagtacatctacgtattagtcatcgctattaccatggtgatgcggttttggcagtacatcaatgggcgtggatagcggtttgactcacggggatttccaagtctccaccccattgacgtcaatgggagtttgttttggcaccaaaatcaacgggactttccaaaatgtcgtaacaactccgccccattgacgcaaatgggcggtaggcgtgtacggtgggaggtctatataagcagagctcgtttagtgaaccggggtctctctggttagaccagatctgagcctgggagctctctggctaactagggaacccactgcttaagcctcaataaagcttgccttgagtgcttcaagtagtgtgtgcccgtctgttgtgtgactctggtaactagagatccctcagacccttttagtcagtgtggaaaatctctagcagtggcgcccgaacagggacttgaaagcgaaagggaaaccagaggagctctctcgacgcaggactcggcttgctgaagcgcgcacggcaagaggcgaggggcggcgactggtgagtacgccaaaaattttgactagcggaggctagaaggagagagatgggtgcgagagcgtcagtattaagcgggggagaattagatcgcgatgggaaaaaattcggttaaggccagggggaaagaaaaaatataaattaaaacatatagtatgggcaagcagggagctagaacgattcgcagttaatcctggcctgttagaaacatcagaaggctgtagacaaatactgggacagctacaaccatcccttcagacaggatcagaagaacttagatcattatataatacagtagcaaccctctattgtgtgcatcaaaggatagagataaaagacaccaaggaagctttagacaagatagaggaagagcaaaacaaaagtaagaccaccgcacagcaagcggccgctgatcttcagacctggaggaggagatatgagggacaattggagaagtgaattatataaatataaagtagtaaaaattgaaccattaggagtagcacccaccaaggcaaagagaagagtggtgcagagagaaaaaagagcagtgggaataggagctttgttccttgggttcttgggagcagcaggaagcactatgggcgcagcgtcaatgacgctgacggtacaggccagacaattattgtctggtatagtgcagcagcagaacaatttgctgagggctattgaggcgcaacagcatctgttgcaactcacagtctggggcatcaagcagctccaggcaagaatcctggctgtggaaagatacctaaaggatcaacagctcctggggatttggggttgctctggaaaactcatttgcaccactgctgtgccttggaatgctagttggagtaataaatctctggaacagatttggaatcacacgacctggatggagtgggacagagaaattaacaattacacaagcttaatacactccttaattgaagaatcgcaaaaccagcaagaaaagaatgaacaagaattattggaattagataaatgggcaagtttgtggaattggtttaacataacaaattggctgtggtatataaaattattcataatgatagtaggaggcttggtaggtttaagaatagtttttgctgtactttctatagtgaatagagttaggcagggatattcaccattatcgtttcagacccacctcccaaccccgaggggacccgacaggcccgaaggaatagaagaagaaggtggagagagagacagagacagatccattcgattagtgaacggatctcgacggtatcggttaacttttaaaagaaaaggggggattggggggtacagtgcaggggaaagaatagtagacataatagcaacagacatacaaactaaagaattacaaaaacaaattacaaaaattcaaaattttatcgatcacgagactagcctcgagaagcttgatatcatggctccggtgcccgtcagtgggcagagcgcacatcgcccacagtccccgagaagttggggggaggggtcggcaattgaaccggtgcctagagaaggtggcgcggggtaaactgggaaagtgatgtcgtgtactggctccgcctttttcccgagggtgggggagaaccgtatataagtgcagtagtcgccgtgaacgttctttttcgcaacgggtttgccgccagaacacaggtgtcgtgacgctcgtcgacacaccggtatgcccggcgtgaccgtgaaggacgtgaaccagcaggagttcgtgagggccctggcagcctttctgaagaagagcggcaagctgaaggtgcccgagtgggtggacacagtgaagctggccaagcacaaggagctggccccttacgatgagaactggttctataccagggcagcctccacagcaaggcacctgtacctgaggggaggagcaggagtgggctctatgaccaagatctatggcggcaggcagcgcaatggcgtgatgccatctcactttagccggggcagcaagtccgtggcaaggagagtgctgcaggccctggagggcctgaagatggtggagaaggaccaggatggcggcagaaagctgacaccacagggacagcgggacctggatagaatcgcaggacaggtggcagcagccaataagaagcactgataggatcccatctagaggatcccccgggctgcaggaattcgagcatcttaccgccatttattcccatatttgttctgtttttcttgatttgggtatacatttaaatgttaataaaacaaaatggtggggcaatcatttacatttttagggatatgtaattactagttcaggtgtattgccacaagacaaacatgttaagaaactttcccgttatttacgctctgttcctgttaatcaacctctggattacaaaatttgtgaaagattgactgatattcttaactatgttgctccttttacgctgtgtggatatgctgctttaatgcctctgtatcatgctattgcttcccgtacggctttcgttttctcctccttgtataaatcctggttgctgtctctttatgaggagttgtggcccgttgtccgtcaacgtggcgtggtgtgctctgtgtttgctgacgcaacccccactggctggggcattgccaccacctgtcaactcctttctgggactttcgctttccccctcccgatcgccacggcagaactcatcgccgcctgccttgcccgctgctggacaggggctaggttgctgggcactgataattccgtggtgttgtcggggaagggcctgctgccggctctgcggcctcttccgcgtcttcgccttcgccctcagacgagtcggatctccctttgggccgcctccccgcctggaattcgagctcggtacctttaagaccaatgacttacaaggcagctgtagatcttagccactttttaaaagaaaaggggggactggaagggctaattcactcccaacgaagacaagatctgctttttgcttgtactgggtctctctggttagaccagatctgagcctgggagctctctggctaactagggaacccactgcttaagcctcaataaagcttgccttgagtgcttcaagtagtgtgtgcccgtctgttgtgtgactctggtaactagagatccctcagacccttttagtcagtgtggaaaatctctagcagtagtagttcatgtcatcttattattcagtatttataacttgcaaagaaatgaatatcagagagtgagaggaacttgtttattgcagcttataatggttacaaataaagcaatagcatcacaaatttcacaaataaagcatttttttcactgcattctagttgtggtttgtccaaactcatcaatgtatcttatcatgtctggctctagctatcccgcccctaactccgcccatcccgcccctaactccgcccatcccgcccctaactccgcccagttccgcccattctccgccccatggctgactaattttttttatttatgcagaggccgaggccgcctcggcctctgagctattccagaagtagtgaggaggcttttttggaggcctagggacgtacccaattcgccctatagtgagtcgtattacgcgcgctcactggccgtcgttttacaacgtcgtgactgggaaaaccctggcgttacccaacttaatcgccttgcagcacatccccctttcgccagctggcgtaatagcgaagaggcccgcaccgatcgcccttcccaacagttgcgcagcctgaatggcgaatgggacgcgccctgtagcggcgcattaagcgcggcgggtgtggtggttacgcgcagcgtgaccgctacacttgccagcgccctagcgcccgctcctttcgctttcttcccttcctttctcgccacgttcgccggctttccccgtcaagctctaaatcgggggctccctttagggttccgatttagtgctttacggcacctcgaccccaaaaaacttgattagggtgatggttcacgtagtgggccatcgccctgatagacggtttttcgccctttgacgttggagtccacgttctttaatagtggactcttgttccaaactggaacaacactcaaccctatctcggtctattcttttgatttataagggattttgccgatttcggcctattggttaaaaaatgagctgatttaacaaaaatttaacgcgaattttaacaaaatcgttccctcaggacgtc

SEQ ID NO: 19 - DNA, 20 bp, Artificial Sequence
  Forward
caggactcggcttgctgaag

SEQ ID NO: 20 - DNA, 20 bp, Artificial Sequence
  Reverse
tcccccgcttaatactgacg

SEQ ID NO: 21 - DNA, 19 bp, Artificial Sequence
  Probe
cgcacggcaagaggcgagg

SEQ ID NO: 22 - DNA, 21 bp, Artificial Sequence
  Forward
gctgtcatctcttgtgggctg

SEQ ID NO: 23 - DNA, 21 bp, Artificial Sequence
  Reverse
actcatgggagctgctggttc

SEQ ID NO: 24 - DNA, 26 bp, Artificial Sequence
  Probe
cctgtcatgcccacacaaatctctcc

SEQ ID NO: 25 - DNA, 20 bp, Artificial Sequence
  Forward
caggactcggcttgctgaag

SEQ ID NO: 26 - DNA, 20 bp, Artificial Sequence
  Reverse
tcccccgcttaatactgacg

SEQ ID NO: 27 - DNA, 19 bp, Artificial Sequence
  Probe
cgcacggcaagaggcgagg

SEQ ID NO: 28 - DNA, 21 bp, Artificial Sequence
  Forward
aaaacgagcagtgacgtgagc

SEQ ID NO: 29 - DNA, 20 bp, Artificial Sequence
  Reverse
ttcagtcatgctgctagcgc

SEQ ID NO: 30 - DNA, 25 bp, Artificial Sequence
  Probe
tgcacggaagcgtctcgtctcagtc

SEQ ID NO: 31-32 - skipped (2 entries)

SEQ ID NO: 33 - DNA, 122 bp, Artificial Sequence
  SV40 Polyadenylation (PolyA) signal sequence
aacttgtttattgcagcttataatggttacaaataaagcaatagcatcacaaatttcacaaataaagcatttttttcactgcattctagttgtggtttgtccaaactcatcaatgtatctta

SEQ ID NO: 34 - DNA, 20 bp, Artificial Sequence
  hGAPDH Fw
gctctctgctcctcctgttc

SEQ ID NO: 35 - DNA, 20 bp, Artificial Sequence
  hGAPDH Rv
acgaccaaatccgttgactc

SEQ ID NO: 36 - DNA, 18 bp, Artificial Sequence
  RPS19 Fw
agccgaggctccaagagt

SEQ ID NO: 37 - DNA, 19 bp, Artificial Sequence
  RPS19 Rv
ccctgaggtgtcagtttgc

SEQ ID NO: 38 - DNA, 20 bp, Artificial Sequence
  CoRPS19 Fw
gtgaaccagcaggagttcgt

SEQ ID NO: 39 - DNA, 18 bp, Artificial Sequence
  CoRPS19 Rv
tcagcttgccgctcttct